European Patent Specification EP 3 562 592 B1, published April 23, 2025. Title: FAST PCR WITH MOLECULAR CROWDING. Applicant: BioFire Defense, LLC Pasko, Christopher P Poritz, Mark A Wernerehl, Aaron. The sequence listing filed with the application follows.

SEQUENCE LISTING (27 sequences)

SEQ ID NO: 1 - DNA, 24 bp, Homo sapiens
cccattcaacgtctacatcgagtc

SEQ ID NO: 2 - DNA, 19 bp, Homo sapiens
tccttctcttgccaggcat

SEQ ID NO: 3 - DNA, 45 bp, Homo sapiens
  mutation (23)..(23): G or A residue
cccattcaacgtctacatcgagtccgatgcctggcaagagaagga

SEQ ID NO: 4 - DNA, 20 bp, Homo sapiens
ctacagtgggagtcacctgc

SEQ ID NO: 5 - DNA, 25 bp, Homo sapiens
ggtactgagctgtgaaagtcaggtt

SEQ ID NO: 6 - DNA, 58 bp, Homo sapiens
  mutation (28)..(28): A or G residue
ctacagtgggagtcacctgcttttgccaaagggaacctgactttcacagctcagtacc

SEQ ID NO: 7 - DNA, 20 bp, Homo sapiens
gggagtcacctgcttttgcc

SEQ ID NO: 8 - DNA, 25 bp, Homo sapiens
tactgagctgtgaaagtcaggttcc

SEQ ID NO: 9 - DNA, 49 bp, Homo sapiens
gggagtcacctgcttttgccaaagggaacctgactttcacagctcagta

SEQ ID NO: 10 - DNA, 34 bp, Homo sapiens
ctctgtgctttctgtatcctcagagtggcattct

SEQ ID NO: 11 - DNA, 28 bp, Homo sapiens
cgtctgctggagtgtgcccaatgctata

SEQ ID NO: 12 - DNA, 60 bp, Homo sapiens
  misc_feature (1)..(41): 5' standard synthetic region
acacacacacacacacacacacacacacacacacacaaaaattcagtggcattaaatacg

SEQ ID NO: 13 - DNA, 67 bp, Homo sapiens
  misc_feature (1)..(50): 5' standard synthetic region
gagagagagagagagagagagagagagagagagagagagagagagaaaaaccagagctaaagggaag

SEQ ID NO: 14 - DNA, 66 bp, Homo sapiens
  misc_feature (1)..(41): 5' standard synthetic region
acacacacacacacacacacacacacacacacacacaaaaagctggtgtctgctatagaactgatt

SEQ ID NO: 15 - DNA, 72 bp, Homo sapiens
  misc_feature (1)..(50): 5' standard synthetic region
gagagagagagagagagagagagagagagagagagagagagagagaaaaagttgccagagctaaagggaagg

SEQ ID NO: 16 - DNA, 41 bp, Artificial Sequence
  Synthetic common primer
acacacacacacacacacacacacacacacacacacaaaaa

SEQ ID NO: 17 - DNA, 50 bp, Artificial Sequence
  Synthetic common primer
gagagagagagagagagagagagagagagagagagagagagagagaaaaa

SEQ ID NO: 18 - DNA, 24 bp, Artificial Sequence
  Synthetic common primer
actcgcacgaactcaccgcactcc

SEQ ID NO: 19 - DNA, 25 bp, Artificial Sequence
  Synthetic common primer
gctctcactcgcactctcacgcaca

SEQ ID NO: 20 - DNA, 100 bp, Artificial Sequence
  Synthetic template
actcgcacgaactcaccgcactccggatggattgtgaagaggcccaagatactggtcatattatcctttgatctagctctcactcgcactctcacgcaca

SEQ ID NO: 21 - DNA, 200 bp, Artificial Sequence
  Synthetic template
actcgcacgaactcaccgcactcctcaatgctgacaaatcgaaagaataggaatagcgtaattactagaggactccaatatagtatattaccctggtgaccgcctgtactgtaggaacactaccgcggttatattgacagcttagcaatctaccctgttgggatctgtttaagtggctctcactcgcactctcacgcaca

SEQ ID NO: 22 - DNA, 300 bp, Artificial Sequence
  Synthetic template
actcgcacgaactcaccgcactccccttcgaatataaagtacgacattactagcaatgacagttccaggatttaagaaagtagtgttccacatcaatgcatatccagtgaaagcataacgtcaaaaaaagcctggcaccgttcgcgatctggacttacttagatttgttgtagtcaagccggctatcagcgatttatcccggaaacacatactagtgagttatttgtatgttacctagaatagctgtcacgaatcactaatacattcacccaccagctctcactcgcactctcacgcaca

SEQ ID NO: 23 - DNA, 400 bp, Artificial Sequence
  Synthetic template
actcgcacgaactcaccgcactcctgaatacaagacgacagtcctgattatattttcatttaattacgccaatttaattatgatgaatattaacggaattaaatatgtattgataagtactaagtaatggtttacccacggcgatctatatgcaagggaaacattaacaaatttaaacatctgatgtggacaaaacttgtaatgtggtatagttaaaaatataggtttcagggacacgtaagtatctatcttgaatgtttaagtaggtcctgtctaccattctgaaatttagaaaatcgcgttcatcgggctgtcggctacacctcagaaaaccatttcgtgttgcacaggaggaactttcgagggttcgtatgagctctcactcgcactctcacgcaca

SEQ ID NO: 24 - DNA, 500 bp, Artificial Sequence
  Synthetic template
actcgcacgaactcaccgcactccaccgcttgacgacgtagggtatttggtatctgaatctactcatttacctacatactgaagattttgcgatcgtctaatatattggactaatgcccgatttctgatcaattactctaggcgatacttcatcgctggccttatttggattttgctcaagtgctaaactctctgcgcgtcaatactagtctgacatcagtcaagacctgctatctgaaaactactagagagatatacctaacaactttagtggataaatcaggtctggagattgtcatataatgccactagggtcagaaggctgtgtcaaagttagtggttagtaggtctccgctctgcggtactattcttatattctcttactatgcatcaaacaaaatagaatgcatagacaaaccgcctgccaagtttacaagataacttgcgtataggtttataagggttcttctgtatcgctctcactcgcactctcacgcaca

SEQ ID NO: 25 - DNA, 31 bp, Homo sapiens
gcttggaagattgctaaaatgatagtcagtg

SEQ ID NO: 26 - DNA, 26 bp, Homo sapiens
ttgatcatactgagcctgctgcataa

SEQ ID NO: 27 - DNA, 60 bp, Homo sapiens
  mutation (34)..(34): A or G residue
gcttggaagattgctaaaatgatagtcagtgacattatgcagcaggctcagtatgatcaa